European Patent Application EP 4 610 272 A1, published September 3, 2025. Title: Novel variant of DNA-binding transcriptional regulator MalT and method for producing L-aromatic amino acid using the same. Applicant: DAESANG CORPORATION. The sequence listing filed with the application follows.

SEQUENCE LISTING (24 sequences)

SEQ ID NO: 1 - DNA, 2706 bp, Escherichia coli
  source 1..2706: mol_type = genomic DNA
atgctgattccgtcaaaactaagtcgtccggttcgactcgaccataccgtggttcgtgagcgcctgctggctaaactttccggcgcgaacaacttccggctggcgctgatcacgagtcctgcgggctacggaaagaccaccctcatttcccagtgggcggcaggcaaaaacgatatcggctggtactcgctggatgaaggtgataaccagcaagagcgtttcgccagctatctcattgccgccgtgcagcaggcaaccaacggtcactgtgcgatatgtgagacgatggcgcaaaaacggcaatatgccagcctgacgtcactcttcgcccagcttttcattgagctggcggaatggcatagcccactttatctggtcatcgatgactatcatctgatcactaatccagtgatccacgagtcaatgcgcttctttattcgccatcaaccagaaaatctcaccctggtggtgttgtcacgcaaccttccgcaactgggcattgccaatctgcgtgttcgtgatcaactgctggaaattggcagtcagcaactggcatttacccatcaggaagcgaagcagttttttgattgccgtctgtcatcgccgattgaagccgcagaaagcagtcggatttgcgatgacgtttccggttgggcgacggcactacagctaatcgccctctccgcccggcagaatacccactcagcccataagtcggcacgccgcctggcgggaatcaatgccagccatctttcggattatctggtcgatgaggttttggataacgtcgatctcgcaacgcgccattttctgttgaaaagcgccattttgcgctcaatgaacgatgccctcatcacccgtgtgaccggcgaagaaaacgggcaaatgcgcctcgaagagattgagcgtcaggggctgtttttacagcggatggatgataccggcgagtggttctgctatcacccgctgtttggtaacttcctgcgccagcgctgccagtgggaactggcggcggagctgccggaaatccaccgtgccgccgcagaaagctggatggcccagggatttcccagcgaagcaattcatcatgcgctggcggcaggcgatgcgctgatgctgcgcgatattctgcttaatcacgcctggagtctgttcaaccatagcgaactgtcgctgctggaagagtcgcttaaggccctgccgtgggacagcttgctggaaaatccgcagttggtgttattgcaggcgtggctgatgcaaagccaacatcgctacggcgaagttaacaccctgctagcccgtgctgaacatgaaatcaaggacatcagagaagacaccatgcacgcagaatttaacgctctgcgcgcccaggtggcgattaacgatggtaatccggatgaagcggaacggctggcaaaactggcactggaagagctgccgccgggctggttctatagccgcattgtggcaacctcggtgctgggtgaagtgctgcactgcaaaggcgaattgacccgctcactggcgctaatgcagcaaaccgaacagatggcacgccagcacgatgtctggcactacgctttgtggagtttaatccagcaaagtgaaattctgtttgcccaagggttcctgcaaaccgcgtgggaaacgcaggaaaaagcattccagctgatcaacgagcagcatctggaacagctgccaatgcatgagtttctggtgcgcattcgtgcgcagctgttatgggcctgggcgcggctggatgaagccgaagcgtcggcgcgtagcgggattgaagtcttgtcgtcttatcagccacagcaacagcttcagtgcctggcaatgttgattcaatgctcgctggcccgtggtgatttagataacgcccgtagccagctgaaccgtctggaaaacctgctggggaatggcaaatatcacagcgactggatctctaacgccaacaaagtccgggtgatttactggcaaatgaccggcgataaagccgccgctgccaactggttgcgtcatacggctaaaccagagtttgcgaacaaccacttcctgcaaggtcaatggcgcaacattgcccgtgcacaaatcttgctgggcgagtttgaaccggcagaaattgttctcgaagaactcaatgaaaatgcccggagtctgcggttgatgagcgatctcaaccgtaacctgttgctgcttaatcaactgtactggcaggccggacgtaaaagtgacgcccagcgcgtgttgctggacgcattaaaactggcgaatcgcaccggatttatcagccattttgtcatcgaaggcgaagcgatggcgcaacaactgcgtcagctgattcagcttaatacgctgccggaactggaacagcatcgcgcgcagcgtattctgcgagaaatcaatcaacatcatcggcataaattcgcccatttcgatgagaatttcgttgaacgtctgctaaatcatcctgaagtacctgaactgatccgcaccagcccgctgacgcaacgtgaatggcaggtactggggctgatctactctggttacagcaatgagcaaattgccggagaactggaagtcgcggcaaccaccatcaaaacgcatatccgcaatctgtatcagaaactcggcgtggcccatcgccaggatgcggtacaacacgcccagcaattgctgaagatgatggggtacggcgtgtaa

SEQ ID NO: 2 - protein, 901 aa, Escherichia coli
MLIPSKLSRPVRLDHTVVRERLLAKLSGANNFRLALITSPAGYGKTTLISQWAAGKNDIGWYSLDEGDNQQERFASYLIAAVQQATNGHCAICETMAQKRQYASLTSLFAQLFIELAEWHSPLYLVIDDYHLITNPVIHESMRFFIRHQPENLTLVVLSRNLPQLGIANLRVRDQLLEIGSQQLAFTHQEAKQFFDCRLSSPIEAAESSRICDDVSGWATALQLIALSARQNTHSAHKSARRLAGINASHLSDYLVDEVLDNVDLATRHFLLKSAILRSMNDALITRVTGEENGQMRLEEIERQGLFLQRMDDTGEWFCYHPLFGNFLRQRCQWELAAELPEIHRAAAESWMAQGFPSEAIHHALAAGDALMLRDILLNHAWSLFNHSELSLLEESLKALPWDSLLENPQLVLLQAWLMQSQHRYGEVNTLLARAEHEIKDIREDTMHAEFNALRAQVAINDGNPDEAERLAKLALEELPPGWFYSRIVATSVLGEVLHCKGELTRSLALMQQTEQMARQHDVWHYALWSLIQQSEILFAQGFLQTAWETQEKAFQLINEQHLEQLPMHEFLVRIRAQLLWAWARLDEAEASARSGIEVLSSYQPQQQLQCLAMLIQCSLARGDLDNARSQLNRLENLLGNGKYHSDWISNANKVRVIYWQMTGDKAAAANWLRHTAKPEFANNHFLQGQWRNIARAQILLGEFEPAEIVLEELNENARSLRLMSDLNRNLLLLNQLYWQAGRKSDAQRVLLDALKLANRTGFISHFVIEGEAMAQQLRQLIQLNTLPELEQHRAQRILREINQHHRHKFAHFDENFVERLLNHPEVPELIRTSPLTQREWQVLGLIYSGYSNEQIAGELEVAATTIKTHIRNLYQKLGVAHRQDAVQHAQQLLKMMGYGV

SEQ ID NO: 3 - DNA, 2706 bp, synthetic construct
  source 1..2706: mol_type = other DNA
atgctgattccgtcaaaactaagtcgtccggttcgactcgaccataccgtggttcgtgagcgcctgctggctaaactttccggcgcgaacaacttccggctggcgctgatcacgagtcctgcgggctacggaaagaccaccctcatttcccagtgggcggcaggcaaaaacgatatcggctggtactcgctggatgaaggtgataaccagcaagagcgtttcgccagctatctcattgccgccgtgcagcaggcaaccaacggtcactgtgcgatatgtgagacgatggcgcaaaaacggcaatatgccagcctgacgtcactcttcgcccagcttttcattgagctggcggaatggcatagcccactttatctggtcatcgatgactatcatctgatcactaatccagtgatccacgagtcaatgcgcttctttattcgccatcaaccagaaaatctcaccctggtggtgttgtcacgcaaccttccgcaactgggcattgccaatctgcgtgttcgtgatcaactgctggaaattggcagtcagcaactggcatttacccatcaggaagcgaagcagttttttgattgccgtctgtcatcgccgattgaagccgcagaaagcagtcggatttgcgatgacgtttccggttgggcgacggcactacagctaatcgccctctccgcccggcagaatacccactcagcccataagtcggcacgccgcctggcgggaatcaatgccagccatctttcggattatctggtcgatgaggttttggataacgtcgatctcgcaacgcgccattttctgttgaaaagcgccattttgcgctcaatgaacgatgccctcatcacccgtgtgaccggcgaagaaaacgggcaaatgcgcctcgaagagattgagcgtcaggggctgtttttacagcggatggatgataccagcgagtggttctgctatcacccgctgtttggtaacttcctgcgccagcgctgccagtgggaactggcggcggagctgccggaaatccaccgtgccgccgcagaaagctggatggcccagggatttcccagcgaagcaattcatcatgcgctggcggcaggcgatgcgctgatgctgcgcgatattctgcttaatcacgcctggagtctgttcaaccatagcgaactgtcgctgctggaagagtcgcttaaggccctgccgtgggacagcttgctggaaaatccgcagttggtgttattgcaggcgtggctgatgcaaagccaacatcgctacggcgaagttaacaccctgctagcccgtgctgaacatgaaatcaaggacatcagagaagacaccatgcacgcagaatttaacgctctgcgcgcccaggtggcgattaacgatggtaatccggatgaagcggaacggctggcaaaactggcactggaagagctgccgccgggctggttctatagccgcattgtggcaacctcggtgctgggtgaagtgctgcactgcaaaggcgaattgacccgctcactggcgctaatgcagcaaaccgaacagatggcacgccagcacgatgtctggcactacgctttgtggagtttaatccagcaaagtgaaattctgtttgcccaagggttcctgcaaaccgcgtgggaaacgcaggaaaaagcattccagctgatcaacgagcagcatctggaacagctgccaatgcatgagtttctggtgcgcattcgtgcgcagctgttatgggcctgggcgcggctggatgaagccgaagcgtcggcgcgtagcgggattgaagtcttgtcgtcttatcagccacagcaacagcttcagtgcctggcaatgttgattcaatgctcgctggcccgtggtgatttagataacgcccgtagccagctgaaccgtctggaaaacctgctggggaatggcaaatatcacagcgactggatctctaacgccaacaaagtccgggtgatttactggcaaatgaccggcgataaagccgccgctgccaactggttgcgtcatacggctaaaccagagtttgcgaacaaccacttcctgcaaggtcaatggcgcaacattgcccgtgcacaaatcttgctgggcgagtttgaaccggcagaaattgttctcgaagaactcaatgaaaatgcccggagtctgcggttgatgagcgatctcaaccgtaacctgttgctgcttaatcaactgtactggcaggccggacgtaaaagtgacgcccagcgcgtgttgctggacgcattaaaactggcgaatcgcaccggatttatcagccattttgtcatcgaaggcgaagcgatggcgcaacaactgcgtcagctgattcagcttaatacgctgccggaactggaacagcatcgcgcgcagcgtattctgcgagaaatcaatcaacatcatcggcataaattcgcccatttcgatgagaatttcgttgaacgtctgctaaatcatcctgaagtacctgaactgatccgcaccagcccgctgacgcaacgtgaatggcaggtactggggctgatctactctggttacagcaatgagcaaattgccggagaactggaagtcgcggcaaccaccatcaaaacgcatatccgcaatctgtatcagaaactcggcgtggcccatcgccaggatgcggtacaacacgcccagcaattgctgaagatgatggggtacggcgtgtaa

SEQ ID NO: 4 - protein, 901 aa, synthetic construct
MLIPSKLSRPVRLDHTVVRERLLAKLSGANNFRLALITSPAGYGKTTLISQWAAGKNDIGWYSLDEGDNQQERFASYLIAAVQQATNGHCAICETMAQKRQYASLTSLFAQLFIELAEWHSPLYLVIDDYHLITNPVIHESMRFFIRHQPENLTLVVLSRNLPQLGIANLRVRDQLLEIGSQQLAFTHQEAKQFFDCRLSSPIEAAESSRICDDVSGWATALQLIALSARQNTHSAHKSARRLAGINASHLSDYLVDEVLDNVDLATRHFLLKSAILRSMNDALITRVTGEENGQMRLEEIERQGLFLQRMDDTSEWFCYHPLFGNFLRQRCQWELAAELPEIHRAAAESWMAQGFPSEAIHHALAAGDALMLRDILLNHAWSLFNHSELSLLEESLKALPWDSLLENPQLVLLQAWLMQSQHRYGEVNTLLARAEHEIKDIREDTMHAEFNALRAQVAINDGNPDEAERLAKLALEELPPGWFYSRIVATSVLGEVLHCKGELTRSLALMQQTEQMARQHDVWHYALWSLIQQSEILFAQGFLQTAWETQEKAFQLINEQHLEQLPMHEFLVRIRAQLLWAWARLDEAEASARSGIEVLSSYQPQQQLQCLAMLIQCSLARGDLDNARSQLNRLENLLGNGKYHSDWISNANKVRVIYWQMTGDKAAAANWLRHTAKPEFANNHFLQGQWRNIARAQILLGEFEPAEIVLEELNENARSLRLMSDLNRNLLLLNQLYWQAGRKSDAQRVLLDALKLANRTGFISHFVIEGEAMAQQLRQLIQLNTLPELEQHRAQRILREINQHHRHKFAHFDENFVERLLNHPEVPELIRTSPLTQREWQVLGLIYSGYSNEQIAGELEVAATTIKTHIRNLYQKLGVAHRQDAVQHAQQLLKMMGYGV

SEQ ID NO: 5 - DNA, 30 bp, synthetic construct
  source 1..30: mol_type = other DNA
caattttattatagtaattgactattatac

SEQ ID NO: 6 - DNA, 40 bp, synthetic construct
  source 1..40: mol_type = other DNA
tcatccatcccaattttattatagtaattgactattatac

SEQ ID NO: 7 - DNA, 40 bp, synthetic construct
  source 1..40: mol_type = other DNA
ggatggatgataccagcgaggttttagagctagaaatagc

SEQ ID NO: 8 - DNA, 30 bp, synthetic construct
  source 1..30: mol_type = other DNA
taccagcgaggttttagagctagaaatagc

SEQ ID NO: 9 - DNA, 21 bp, synthetic construct
  source 1..21: mol_type = other DNA
gagcctgtcggcctacctgct

SEQ ID NO: 10 - DNA, 20 bp, synthetic construct
  source 1..20: mol_type = other DNA
cggccggcatgagcctgtcg

SEQ ID NO: 11 - DNA, 30 bp, synthetic construct
  source 1..30: mol_type = other DNA
atgccggccgacccatcaggaagcgaagca

SEQ ID NO: 12 - DNA, 23 bp, synthetic construct
  source 1..23: mol_type = other DNA
acccatcaggaagcgaagcagtt

SEQ ID NO: 13 - DNA, 25 bp, synthetic construct
  source 1..25: mol_type = other DNA
atccgctgtaaaaacagcccctgac

SEQ ID NO: 14 - DNA, 25 bp, synthetic construct
  source 1..25: mol_type = other DNA
ggtatcatccatccgctgtaaaaac

SEQ ID NO: 15 - DNA, 30 bp, synthetic construct
  source 1..30: mol_type = other DNA
ggatgataccagcgagtggttctgctatca

SEQ ID NO: 16 - DNA, 25 bp, synthetic construct
  source 1..25: mol_type = other DNA
agcgagtggttctgctatcacccgc

SEQ ID NO: 17 - DNA, 25 bp, synthetic construct
  source 1..25: mol_type = other DNA
gttaacttcgccgtagcgatgttgg

SEQ ID NO: 18 - DNA, 25 bp, synthetic construct
  source 1..25: mol_type = other DNA
ctagcagggtgttaacttcgccgta

SEQ ID NO: 19 - DNA, 33 bp, synthetic construct
  source 1..33: mol_type = other DNA
accctgctaggagctcctgaaaatctcgataac

SEQ ID NO: 20 - DNA, 23 bp, synthetic construct
  source 1..23: mol_type = other DNA
gagctcctgaaaatctcgataac

SEQ ID NO: 21 - DNA, 20 bp, synthetic construct
  source 1..20: mol_type = other DNA
cattgccaatctgcgtgttc

SEQ ID NO: 22 - DNA, 20 bp, synthetic construct
  source 1..20: mol_type = other DNA
accatcgttaatcgccacct

SEQ ID NO: 23 - DNA, 3234 bp, synthetic construct
  source 1..3234: mol_type = other DNA
tttccataggctccgcccccctgacgagcatcacaaaaatcgacgctcaagtcagaggtggcgaaacccgacaggactataaagataccaggcgtttccccctggaagctccctcgtgcgctctcctgttccgaccctgccgcttaccggatacctgtccgcctttctcccttcgggaagcgtggcgctttctcatagctcacgctgtaggtatctcagttcggtgtaggtcgttcgctccaagctgggctgtgtgcacgaaccccccgttcagcccgaccgctgcgccttatccggtaactatcgtcttgagtccaacccggtaagacacgacttatcgccactggcagcagccactggtaacaggattagcagagcgaggtatgtaggcggtgctacagagttcttgaagtggtggcctaactacggctacactagaaggacagtatttggtatctgcgctctgctgaagccagttaccttcggaaaaagagttggtagctcttgatccggcaaacaaaccaccgctggtagcggtggtttttttgtttgcaagcagcagattacgcgcagaaaaaaaggatctcaagaagatcctttgatcttttctacggggtctgacgctcagtggaacgaaaactcacgttaagggattttggtcatgagattatcaaaaaggatcttcacctagatccttttaaattaaaaatgaagttttaaatcaatctaaagtatatatgagtaaacttggtctgacagttaaaagattgacagtataatagtcaattactataataaaattgatgcgcaggtgaaacacctgctgcagttttagagctagaaatagcaagttaaaataaggctagtccgttatcaacttgaaaaagtggcaccgagtcggtgctttttttcgttttccgggacgccctcgcggacgtgctcatagtccacgacgcccgtgattttgtagccctggccgacggccagcaggtaggccgacaggctcatgccggccggagctcctgaaaatctcgataactcaaaaaatacgcccggtagtgatcttatttcattatggtgaaagttggaacctcttaggatcctctagatttaagaaggagatatacataaaactccttctgagctagttctctagcattctattattttgattcgacaccttaataatagcagaaggagtttttacctgtcaaagaaccatcaaacccttgatacacaaggctttgacctaattttgaaaaatgatgttgtttctatatagtatcaagataagaaagaaaaggatttttcgctacgctcaaatcctttcccgtcacgggcttctcagggcgttttatggcgggtctgctatgtggtgctatctgactttttgctgttcagcagttcctgccctctgattttccagtctgaccacttcggattatcccgtgacaggtcattcagactggctaatgcacccagtaaggcagcggtatcatcaacggggtctgacgctcagtggaacgaaaactcacgttaagggattttggtcatgagattatcaaaaaggatcttcacctagatccttttaaattaaaaatgaagttttaaatcaatctaaagtatatatgagtaaacttggtctgacagttaccaatgcttaatcagtgaggcacctatctcagcgatctgtctatttcgttcatccatagttgcctgactccccgtcgtgtagataactacgatacgggagggcttaccatctggccccagtgctgcaatgataccgcgagacccacgctcaccggctccagatttatcagcaataaaccagccagccggaagggccgagcgcagaagtggtcctgcaactttatccgcctccatccagtctattaattgttgccgggaagctagagtaagtagttcgccagttaatagtttgcgcaacgttgttgccattgctacaggcatcgtggtgtcacgctcgtcgtttggtatggcttcattcagctccggttcccaacgatcaaggcgagttacatgatcccccatgttgtgcaaaaaagcggttagctccttcggtcctccgatcgttgtcagaagtaagttggccgcagtgttatcactcatggttatggcagcactgcataattctcttactgtcatgccatccgtaagatgcttttctgtgactggtgagtactcaaccaagtcattctgagaatagtgtatgcggcgaccgagttgctcttgcccggcgtcaatacgggataataccgcgccacatagcagaactttaaaagtgctcatcattggaaaacgttcttcggggcgaaaactctcaaggatcttaccgctgttgagatccagttcgatgtaacccactcgtgcacccaactgatcttcagcatcttttactttcaccagcgtttctgggtgagcaaaaacaggaaggcaaaatgccgcaaaaaagggaataagggcgacacggaaatgttgaatactcatactcttcctttttcaatattattgaagcatttatcagggttattgtctcatgagcggatacatatttgaatgtatttagaaaaataaacaaataggggttccgcgcacatttccccgaaaagtgccaccaaaaaaacacaaaagaccacattttttaatgtggtctttattcttcaactaaagcacccattagttcaacaaacgaaaattggataaagtgggatatttttaaaatatatatttatgttacagtaagctgcctcgcgcgtttcggtgatgacggtgaaaacctctgacacatgcagctcccggagacggtcacagcttgtctgtaagcggatgccgggagcagacaagcccgtcagggcgcgtcagcgggtgttggcgggtgtcggggcgcagccatgacccagtcacgtagcgatagcggagtgtatactggcttaactatgcggcatcagagcagattgtactgagagtgcaccatatgcggtgtgaaataccgcacagatgcgtaaggagaaaataccgcatcaggcgctcttccgcttcctcgctcactgactcgctgcgctcggtcgttcggctgcggcgagcggtatcagctcactcaaaggcggtaatacggttatccacagaatcaggggataacgcaggaaagaacatgtgagcaaaaggccagcaaaaggccaggaaccgtaaaaaggccgcgttgctggcgtt

SEQ ID NO: 24 - DNA, 9656 bp, synthetic construct
  source 1..9656: mol_type = other DNA
aaagccatgacaaaaacgcgtaacaaaagtgtctataatcacggcagaaaagtccacattgattatttgcacggcgtcacactttgctatgccatagcatttttatccataagattagcggatcctacctgacgctttttatcgcaactctctactgtttctccatacccgtttttttgggaattcgagctctaaggaggttataaaaaatggatattaatactgaaactgagatcaagcaaaagcattcactaaccccctttcctgttttcctaatcagcccggcatttcgcgggcgatattttcacagctatttcaggagttcagccatgaacgcttattacattcaggatcgtcttgaggctcagagctgggcgcgtcactaccagcagctcgcccgtgaagagaaagaggcagaactggcagacgacatggaaaaaggcctgccccagcacctgtttgaatcgctatgcatcgatcatttgcaacgccacggggccagcaaaaaatccattacccgtgcgtttgatgacgatgttgagtttcaggagcgcatggcagaacacatccggtacatggttgaaaccattgctcaccaccaggttgatattgattcagaggtataaaacgaatgagtactgcactcgcaacgctggctgggaagctggctgaacgtgtcggcatggattctgtcgacccacaggaactgatcaccactcttcgccagacggcatttaaaggtgatgccagcgatgcgcagttcatcgcattactgatcgttgccaaccagtacggccttaatccgtggacgaaagaaatttacgcctttcctgataagcagaatggcatcgttccggtggtgggcgttgatggctggtcccgcatcatcaatgaaaaccagcagtttgatggcatggactttgagcaggacaatgaatcctgtacatgccggatttaccgcaaggaccgtaatcatccgatctgcgttaccgaatggatggatgaatgccgccgcgaaccattcaaaactcgcgaaggcagagaaatcacggggccgtggcagtcgcatcccaaacggatgttacgtcataaagccatgattcagtgtgcccgtctggccttcggatttgctggtatctatgacaaggatgaagccgagcgcattgtcgaaaatactgcatacactgcagaacgtcagccggaacgcgacatcactccggttaacgatgaaaccatgcaggagattaacactctgctgatcgccctggataaaacatgggatgacgacttattgccgctctgttcccagatatttcgccgcgacattcgtgcatcgtcagaactgacacaggccgaagcagtaaaagctcttggattcctgaaacagaaagccgcagagcagaaggtggcagcatgacaccggacattatcctgcagcgtaccgggatcgatgtgagagctgtcgaacagggggatgatgcgtggcacaaattacggctcggcgtcatcaccgcttcagaagttcacaacgtgatagcaaaaccccgctccggaaagaagtggcctgacatgaaaatgtcctacttccacaccctgcttgctgaggtttgcaccggtgtggctccggaagttaacgctaaagcactggcctggggaaaacagtacgagaacgacgccagaaccctgtttgaattcacttccggcgtgaatgttactgaatccccgatcatctatcgcgacgaaagtatgcgtaccgcctgctctcccgatggtttatgcagtgacggcaacggccttgaactgaaatgcccgtttacctcccgggatttcatgaagttccggctcggtggtttcgaggccataaagtcagcttacatggcccaggtgcagtacagcatgtgggtgacgcgaaaaaatgcctggtactttgccaactatgacccgcgtatgaagcgtgaaggcctgcattatgtcgtgattgagcgggatgaaaagtacatggcgagttttgacgagatcgtgccggagttcatcgaaaaaatggacgaggcactggctgaaattggttttgtatttggggagcaatggcgatgagatctaaagaggagaaaggatctatggataagaaatactcaataggcttagatatcggcacaaatagcgtcggatgggcggtgatcactgatgaatataaggttccgtctaaaaagttcaaggttctgggaaatacagaccgccacagtatcaaaaaaaatcttataggggctcttttatttgacagtggagagacagcggaagcgactcgtctcaaacggacagctcgtagaaggtatacacgtcggaagaatcgtatttgttatctacaggagattttttcaaatgagatggcgaaagtagatgatagtttctttcatcgacttgaagagtcttttttggtggaagaagacaagaagcatgaacgtcatcctatttttggaaatatagtagatgaagttgcttatcatgagaaatatccaactatctatcatctgcgaaaaaaattggtagattctactgataaagcggatttgcgcttaatctatttggccttagcgcatatgattaagtttcgtggtcattttttgattgagggagatttaaatcctgataatagtgatgtggacaaactatttatccagttggtacaaacctacaatcaattatttgaagaaaaccctattaacgcaagtggagtagatgctaaagcgattctttctgcacgattgagtaaatcaagacgattagaaaatctcattgctcagctccccggtgagaagaaaaatggcttatttgggaatctcattgctttgtcattgggtttgacccctaattttaaatcaaattttgatttggcagaagatgctaaattacagctttcaaaagatacttacgatgatgatttagataatttattggcgcaaattggagatcaatatgctgatttgtttttggcagctaagaatttatcagatgctattttactttcagatatcctaagagtaaatactgaaataactaaggctcccctatcagcttcaatgattaaacgctacgatgaacatcatcaagacttgactcttttaaaagctttagttcgacaacaacttccagaaaagtataaagaaatcttttttgatcaatcaaaaaacggatatgcaggttatattgatgggggagctagccaagaagaattttataaatttatcaaaccaattttagaaaaaatggatggtactgaggaattattggtgaaactaaatcgtgaagatttgctgcgcaagcaacggacctttgacaacggctctattccccatcaaattcacttgggtgagctgcatgctattttgagaagacaagaagacttttatccatttttaaaagacaatcgtgagaagattgaaaaaatcttgacttttcgaattccttattatgttggtccattggcgcgtggcaatagtcgttttgcatggatgactcggaagtctgaagaaacaattaccccatggaattttgaagaagttgtcgataaaggtgcttcagctcaatcatttattgaacgcatgacaaactttgataaaaatcttccaaatgaaaaagtactaccaaaacatagtttgctttatgagtattttacggtttataacgaattgacaaaggtcaaatatgttactgaaggaatgcgaaaaccagcatttctttcaggtgaacagaagaaagccattgttgatttactcttcaaaacaaatcgaaaagtaaccgttaagcaattaaaagaagattatttcaaaaaaatagaatgttttgatagtgttgaaatttcaggagttgaagatagatttaatgcttcattaggtacctaccatgatttgctaaaaattattaaagataaagattttttggataatgaagaaaatgaagatatcttagaggatattgttttaacattgaccttatttgaagatagggagatgattgaggaaagacttaaaacatatgctcacctctttgatgataaggtgatgaaacagcttaaacgtcgccgttatactggttggggacgtttgtctcgaaaattgattaatggtattagggataagcaatctggcaaaacaatattagattttttgaaatcagatggttttgccaatcgcaattttatgcagctgatccatgatgatagtttgacatttaaagaagacattcaaaaagcacaagtgtctggacaaggcgatagtttacatgaacatattgcaaatttagctggtagccctgctattaaaaaaggtattttacagactgtaaaagttgttgatgaattggtcaaagtaatggggcggcataagccagaaaatatcgttattgaaatggcacgtgaaaatcagacaactcaaaagggccagaaaaattcgcgagagcgtatgaaacgaatcgaagaaggtatcaaagaattaggaagtcagattcttaaagagcatcctgttgaaaatactcaattgcaaaatgaaaagctctatctctattatctccaaaatggaagagacatgtatgtggaccaagaattagatattaatcgtttaagtgattatgatgtcgatcacattgttccacaaagtttccttaaagacgattcaatagacaataaggtcttaacgcgttctgataaaaatcgtggtaaatcggataacgttccaagtgaagaagtagtcaaaaagatgaaaaactattggagacaacttctaaacgccaagttaatcactcaacgtaagtttgataatttaacgaaagctgaacgtggaggtttgagtgaacttgataaagctggttttatcaaacgccaattggttgaaactcgccaaatcactaagcatgtggcacaaattttggatagtcgcatgaatactaaatacgatgaaaatgataaacttattcgagaggttaaagtgattaccttaaaatctaaattagtttctgacttccgaaaagatttccaattctataaagtacgtgagattaacaattaccatcatgcccatgatgcgtatctaaatgccgtcgttggaactgctttgattaagaaatatccaaaacttgaatcggagtttgtctatggtgattataaagtttatgatgttcgtaaaatgattgctaagtctgagcaagaaataggcaaagcaaccgcaaaatatttcttttactctaatatcatgaacttcttcaaaacagaaattacacttgcaaatggagagattcgcaaacgccctctaatcgaaactaatggggaaactggagaaattgtctgggataaagggcgagattttgccacagtgcgcaaagtattgtccatgccccaagtcaatattgtcaagaaaacagaagtacagacaggcggattctccaaggagtcaattttaccaaaaagaaattcggacaagcttattgctcgtaaaaaagactgggatccaaaaaaatatggtggttttgatagtccaacggtagcttattcagtcctagtggttgctaaggtggaaaaagggaaatcgaagaagttaaaatccgttaaagagttactagggatcacaattatggaaagaagttcctttgaaaaaaatccgattgactttttagaagctaaaggatataaggaagttaaaaaagacttaatcattaaactacctaaatatagtctttttgagttagaaaacggtcgtaaacggatgctggctagtgccggagaattacaaaaaggaaatgagctggctctgccaagcaaatatgtgaattttttatatttagctagtcattatgaaaagttgaagggtagtccagaagataacgaacaaaaacaattgtttgtggagcagcataagcattatttagatgagattattgagcaaatcagtgaattttctaagcgtgttattttagcagatgccaatttagataaagttcttagtgcatataacaaacatagagacaaaccaatacgtgaacaagcagaaaatattattcatttatttacgttgacgaatcttggagctcccgctgcttttaaatattttgatacaacaattgatcgtaaacgatatacgtctacaaaagaagttttagatgccactcttatccatcaatccatcactggtctttatgaaacacgcattgatttgagtcagctaggaggtgactaacgcatcctcacgataatatccgggtaggcgcaatcactttcgtctactccgttacaaagcgaggctgggtatttcccggcctttctgttatccgaaatccactgaaagcacagcggctggctgaggagataaataataaacgaggggctgtatgcacaaagcatcttctgttgagttaagaacgagtatcgagatggcacatagccttgctcaaattggaatcaggtttgtgccaataccagtagaaacagacgaagaatccatgggtatggacagttttccctttgatatgtaacggtgaacagttgttctacttttgtttgttagtcttgatgcttcactgatagatacaagagccaaatctagtaatattttatctgattaataagatgatcttcttgagatcgttttggtctgcgcgtaatctcttgctctgaaaacgaaaaaaccgccttgcagggcggtttttcgaaggttctctgagctaccaactctttgaaccgaggtaactggcttggaggagcgcagtcaccaaaacttgtcctttcagtttagccttaaccggcgcatgacttcaagactaactcctctaaatcaattaccagtggctgctgccagtggtgcttttgcatgtctttccgggttggactcaagacgatagttaccggataaggcgcagcggtcggactgaacggggggttcgtgcatacagtccagcttggagcgaactgcctacccggaactgagtgtcaggcgtggaatgagacaaacgcggccataacagcggaatgacaccggtaaaccgaaaggcaggaacaggagagcgcacgagggagccgccagggggaaacgcctggtatctttatagtcctgtcgggtttcgccaccactgatttgagcgtcagatttcgtgatgcttgtcaggggggcggagcctatggaaaaacggctttgccgcggccccgctgaatattccttttgtctccgaccatcaggcacctgagtcgctgtctttttcgtgacattcagttcgctgcgctcacggctctggcagtgaatgggggtaaatggcactacaggcgccttttatggattcatgcaaggaaactacccataatacaagaaaagatgtggtctttattcttcaactaaagcacccattagttcaacaaacgaaaattggataaagtgggatatttttaaaatatatatttatgttacctggcagagcctgtactttttacagtcggttttctaatgtcactaacctgccccgttagtcgccatttgcatcgatttattatgacaacttgacggctacatcattcactttttcttcacaaccggcacggaactcgctcgggctggccccggtgcattttttaaatacccgcgagaaatagagttgatcgtcaaaaccaacattgcgaccgacggtggcgataggcatccgggtggtgctcaaaagcagcttcgcctggctgatacgttggtcctcgcgccagcttaagacgctaatccctaactgctggcggaaaagatgtgacagacgcgacggcgacaagcaaacatgctgtgcgacgctggcgatatcaaaattgctgtctgccaggtgatcgctgatgtactgacaagcctcgcgtacccgattatccatcggtggatggagcgactcgttaatcgcttccatgcgccgcagtaacaattgctcaagcagatttatcgccagcagctccgaatagcgcccttccccttgcccggcgttaatgatttgcccaaacaggtcgctgaaatgcggctggtgcgcttcatccgggcgaaagaaccccgtattggcaaatattgacggccagttaagccattcatgccagtaggcgcgcggacgaaagtaaacccactggtgataccattcgcgagcctccggatgacgaccgtagtgatgaatctctcctggcgggaacagcaaaatatcacccggtcggcaaacaaattctcgtccctgatttttcaccaccccctgaccgcgaatggtgagattgagaatataacctttcattcccagcggtcggtcgataaaaaaatcgagataaccgttggcctcaatcggcgttaaacccgccaccagatgggcattaaacgagtatcccggcagcaggggatcattttgcgcttcagccatacttttcatactcccgccattcagagaagaaaccaattgtccatattgcatcagacattgccgtcactgcgtcttttactggctcttctcgctaaccaaaccggtaaccccgcttattaaaagcattctgtaacaaagcgggaccagtaatagaaagtgagggagccacggttgatgagagctttgttgtaggtggaccagttggtgattttgaacttttgctttgccacggaacggtctgcgttgtcgggaagatgcgtgatctgatccttcaactcagcaaaagttcgatttattcaacaaagccacgttgtgtctcaaaatctctgatgttacattgcacaagataaaaatatatcatcatgaacaataaaactgtctgcttacataaacagtaatacaaggggtgttatgagccatattcaacgggaaacgtcttgctcgaggccgcgattaaattccaacatggatgctgatttatatgggtataaatgggctcgcgataatgtcgggcaatcaggtgcgacaatctatcgattgtatgggaagcccgatgcgccagagttgtttctgaaacatggcaaaggtagcgttgccaatgatgttacagatgagatggtcagactaaactggctgacggaatttatgcctcttccgaccatcaagcattttatccgtactcctgatgatgcatggttactcaccactgcgatccccgggaaaacagcattccaggtattagaagaatatcctgattcaggtgaaaatattgttgatgcgctggcagtgttcctgcgccggttgcattcgattcctgtttgtaattgtccttttaacagcgatcgcgtatttcgtctcgctcaggcgcaatcacgaatgaataacggtttggttgatgcgagtgattttgatgacgagcgtaatggctggcctgttgaacaagtctggaaagaaatgcataagcttttgccattctcaccggattcagtcgtcactcatggtgatttctcacttgataaccttatttttgacgaggggaaattaataggttgtattgatgttggacgagtcggaatcgcagaccgataccaggatcttgccatcctatggaactgcctcggtgagttttctccttcattacagaaacggctttttcaaaaatatggtattgataatcctgatatgaataaattgcagtttcatttgatgctcgatgagtttttctaatcagaattggttaattggttgtaaca